European Patent Application EP 4 119 679 A1, published January 18, 2023. Title: Polynucleotide Adapter Design for Reduced Bias. Applicant: New England Biolabs, Inc. Application Not yet assigned. The sequence listing filed with the application follows.

SEQUENCE LISTING (5 sequences)

SEQ ID NO: 1 - DNA, 24 bp, Artificial Sequence
  Synthetic construct
  misc_feature (22)..(24): 3InvdT
agatcggaagagcacacgtctttt

SEQ ID NO: 2 - DNA, 30 bp, Artificial Sequence
  Synthetic construct
  misc_feature (21)..(21): n at position 21 is ideoxyU
  misc_feature (22)..(22): n at position 22 is a, or t, or g, or c, where 25 percent of the DNA molecues in the population have a, 25 percent have t, 25 percent have g and 25 percent have c.
  misc_feature (23)..(27): n is a, c, g, or t
agacgtgtgctcttccgatcnnnnnnnttt

SEQ ID NO: 3 - RNA, 26 nt, Artificial Sequence
  Synthetic construct
guucagaguucuacaguccgacgauc

SEQ ID NO: 4 - RNA, 32 nt, Artificial Sequence
  Synthetic construct
  misc_feature (1)..(1): n at position 1 is a, or t, or g, or c where 25 percent of the DNA molecues in the population have a, 25 percent have t, 25 percent have g and 25 percent have c.
  misc_feature (2)..(6): n is a, c, g, or u
nnnnnngaucgucggacuguagaacucugaac

SEQ ID NO: 5 - RNA, 35 nt, Artificial Sequence
  Synthetic construct
  modified_base (1)..(6)
  misc_feature (1)..(1): n at position 1 is a, or t, or g, or c where 25 percent of the DNA molecues in the population have a, 25 percent have t, 25 percent have g and 25 percent have c.
  misc_feature (2)..(6): n is a, c, g, or u
  misc_feature (33)..(35): n is t
  misc_feature (33)..(35): n is 3InvdT
nnnnnngaucgucggacuguagaacucugaacnnn